European Patent Specification EP 3 889 173 B1, published July 5, 2023. Title: Optimized Factor VIII Gene. Applicant: Biogen MA Inc. Application EP14751254.5. The sequence listing filed with the application follows.

SEQUENCE LISTING (51 sequences)

SEQ ID NO: 1 - DNA, 4404 bp, Artificial Sequence
  optimized BDD FVIII
cgtacggccgccaccatgcagattgagctgtctacttgctttttcctgtgcctgctgaggttttgcttttccgctacacgaaggtattatctgggggctgtggaactgtcttgggattacatgcagagtgacctgggagagctgccagtggacgcaaggtttccccctagagtccctaagtcattccccttcaacactagcgtggtctacaagaaaacactgttcgtggagtttactgatcacctgttcaacatcgcaaagcctaggccaccctggatgggactgctggggccaacaatccaggccgaggtgtacgacaccgtggtcattacacttaagaacatggcctcacaccccgtgagcctgcatgctgtgggcgtcagctactggaaggcttccgaaggagcagagtatgacgatcagacttcccagagagaaaaagaggacgataaggtgtttcctggcggatctcatacctacgtgtggcaggtcctgaaagagaatggccctatggcctccgaccctctgtgcctgacctactcttatctgagtcacgtggacctggtcaaggatctgaacagcggcctgatcggagccctgctggtgtgcagggaaggaagcctggctaaggagaaaacccagacactgcataagttcattctgctgttcgccgtgtttgacgaagggaaatcatggcacagcgagacaaagaatagtctgatgcaggacagggatgccgcttcagccagagcttggcccaaaatgcacactgtgaacggctacgtcaatcgctcactgcctgggctgatcggctgccaccgaaagagcgtgtattggcatgtcatcgggatgggcaccacacctgaagtgcactccattttcctggagggacatacctttctggtccgcaaccaccgacaggcttccctggagatctctccaattaccttcctgacagcacagactctgctgatggacctggggcagttcctgctgttttgccacatcagctcccaccagcatgatggcatggaggcttacgtgaaagtggactcttgtcccgaggaacctcagctgcggatgaagaacaatgaggaagcagaagactatgacgatgacctgaccgactccgagatggatgtggtccgattcgatgacgataacagcccctcctttatccagattagatctgtggccaagaaacaccctaagacatgggtccattacatcgcagccgaggaagaggactgggattatgcaccactggtgctggcaccagacgatcgctcctacaaatctcagtatctgaacaatgggccacagaggattggcagaaagtacaagaaagtgcggttcatggcatataccgatgagaccttcaagactcgcgaagccatccagcacgagagcggcatcctgggaccactgctgtacggagaagtgggagacaccctgctgatcattttcaagaaccaggccagccggccttacaatatctatccacatgggattacagatgtgcgccctctgtacagcaggagactgccaaagggcgtcaaacacctgaaggacttcccaatcctgcccggagaaatcttcaagtacaagtggactgtcaccgtcgaggatggccccactaagagcgaccctcggtgcctgacccgctactattctagtttcgtgaatatggaaagagatctggcaagcggactgatcggaccactgctgatttgttacaaagagagcgtggatcagagaggcaaccagatcatgtccgacaagcggaatgtgattctgttcagtgtctttgacgaaaacaggtcatggtacctgaccgagaacatccagagattcctgcctaatccagctggggtgcagctggaagatcctgagtttcaggcatctaacatcatgcatagtattaatggctacgtgttcgacagtttgcagctgagcgtgtgcctgcacgaggtcgcttactggtatatcctgagcattggggcacagacagatttcctgagcgtgttcttttccggctacacttttaagcataaaatggtctatgaggacacactgactctgttccccttcagcggcgaaaccgtgtttatgagcatggagaatcccggactgtggattctggggtgccacaacagcgatttcagaaatcgcggaatgactgccctgctgaaagtgtcaagctgtgacaagaacaccggggactactatgaagattcatacgaggacatcagcgcatatctgctgtccaaaaacaatgccattgaaccccggtcttttagtcagaatcctccagtgctgaagcggcaccagcgcgagatcacccgcactaccctgcagagtgatcaggaagagatcgactacgacgatacaatttctgtggaaatgaagaaagaggacttcgatatctatgacgaagatgagaaccagagtcctcgatcattccagaagaaaaccaggcattactttattgccgcagtggagcggctgtgggattatggcatgtcctctagtcctcacgtgctgcgaaatagggcccagtcaggaagcgtcccacagttcaagaaagtggtcttccaggagtttacagacgggtcctttactcagccactgtacaggggcgaactgaacgagcacctgggactgctggggccctatatcagagcagaagtggaggataacattatggtcaccttcagaaatcaggcctctcggccttacagtttttattcaagcctgatctcttacgaagaggaccagcgacagggagctgaaccacgaaaaaacttcgtgaagcctaatgagaccaaaacatacttttggaaggtgcagcaccatatggccccaacaaaagacgagttcgattgcaaggcatgggcctatttttctgacgtggatctggagaaggacgtgcacagtggcctgattggcccactgctggtgtgccatactaacaccctgaatccagcccacggccggcaggtcactgtccaggagttcgctctgttctttaccatctttgatgagacaaagagctggtacttcaccgaaaacatggagcgaaattgcagggctccatgtaacattcagatggaagaccccacattcaaggagaactaccgctttcatgctatcaatggatacatcatggatactctgcccgggctggtcatggcacaggaccagagaatccggtggtatctgctgagcatgggcagcaacgagaatatccactcaattcatttcagcgggcacgtgtttactgtcaggaagaaagaagagtacaagatggccctgtacaacctgtatcccggcgtgttcgaaaccgtcgagatgctgcctagcaaggccggaatctggagagtggaatgcctgattggagagcacctgcatgctgggatgtctaccctgtttctggtgtacagtaataagtgtcagacacccctgggaatggcatccgggcatatcagggatttccagattaccgcatctggacagtacggacagtgggcacctaagctggctagactgcactattccggatctatcaacgcttggtccacaaaagagcctttctcttggattaaggtggacctgctggccccaatgatcattcatggcatcaaaactcagggagctcggcagaagttctcctctctgtacatctcacagtttatcatcatgtacagcctggatgggaagaaatggcagacataccgcggcaatagcacaggaactctgatggtgttctttggcaacgtggacagcagcggaatcaagcacaacattttcaatccccctatcattgctagatacatccggctgcacccaacccattattctattcgaagtacactgaggatggaactgatgggatgcgatctgaacagttgttcaatgcccctggggatggagtccaaggcaatctctgacgcccagattaccgctagctcctacttcactaatatgtttgctacctggagcccttccaaagcaagactgcacctgcaaggccgcagcaacgcatggcgaccacaggtgaacaatcccaaggagtggttgcaggtcgattttcagaaaactatgaaggtgaccggggtcacaactcagggcgtgaaaagtctgctgacctcaatgtacgtcaaggagttcctgatctctagttcacaggacggacatcagtggacactgttctttcagaacgggaaggtgaaagtcttccagggcaatcaggattcctttacacctgtggtcaacagtctagaccctccactgctgaccagatacctgagaatccaccctcagtcctgggtgcaccagattgccctgagaatggaagtgctgggatgcgaggcccaggatctgtactgataactcgagtcgacc

SEQ ID NO: 2 - DNA, 4419 bp, Artificial Sequence
  optimized BDD FVIII
ggcgcgcccgtacggccgccaccatgcagatcgagctgtctacctgcttcttcctgtgcctgctgcggttctgcttcagcgccacccggcggtactacctgggcgccgtggaactgagctgggactacatgcagagcgacctgggggagctgcccgtggacgccagattccccccaagagtgcccaagagcttccccttcaacacctccgtggtgtacaagaaaaccctgttcgtcgagttcaccgaccacctgttcaatatcgccaagcccagacccccctggatgggcctgctgggccctacaatccaggccgaggtgtacgacaccgtggtcatcacccttaagaacatggccagccaccccgtgtccctgcacgccgtgggcgtgtcctactggaaggcctctgagggcgctgagtacgacgaccagaccagccagcgcgagaaagaggacgacaaagtctttcctggcggcagccatacctacgtgtggcaggtcctgaaagaaaacggccctatggcctccgaccccctgtgcctgacctacagctacctgagccacgtggacctggtcaaggacctgaacagcggcctgattggcgccctgctcgtgtgtagagagggcagcctcgccaaagagaaaacccagaccctgcacaagttcatcctgctgttcgccgtgttcgacgagggcaagagctggcacagcgagacaaagaacagcctgatgcaggaccgggacgccgcctctgccagagcctggcctaagatgcacaccgtgaacggctacgtgaacagaagcctgcccggactgatcggctgccaccggaagtccgtgtactggcacgtgatcggcatgggcaccacccccgaggtgcacagcatctttctggaaggccacaccttcctcgtgcggaaccacagacaggccagcctggaaatcagccctatcaccttcctgaccgcccagacactgctgatggacctgggccagttcctgctgttttgccacatcagcagccaccagcacgacggcatggaagcctacgtgaaggtggacagctgccccgaggaaccccagctgcggatgaagaacaacgaggaagccgaggactacgacgacgacctgaccgacagcgagatggacgtcgtgcgcttcgacgacgacaacagccccagcttcatccagatcagaagcgtggccaagaagcaccccaagacctgggtgcactatatcgccgccgaggaagaggactgggactacgcccctctggtgctggcccccgacgacagaagctacaagagccagtacctgaacaatggcccccagcggatcggccggaagtacaagaaagtgcggttcatggcctacaccgacgagacattcaagaccagagaggccatccagcacgagagcggcatcctgggccccctgctgtatggcgaagtgggcgacaccctgctgatcatcttcaagaaccaggccagccggccctacaacatctacccccacggcatcaccgacgtgcggcccctgtacagcagacggctgcccaagggcgtgaagcacctgaaggacttccccatcctgcccggcgagatcttcaagtacaagtggaccgtgaccgtggaagatggccccaccaagagcgaccccagatgcctgacccggtactacagcagcttcgtgaacatggaacgggacctggcctccgggctgatcggccctctgctgatctgctacaaagaaagcgtggaccagcggggcaaccagatcatgagcgacaagcggaacgtgatcctgttcagcgtgttcgatgagaatcggtcctggtacctgaccgagaatatccagcggttcctgcccaaccctgccggcgtgcagctggaagatcccgagttccaggccagcaacatcatgcactccatcaatggctacgtgttcgacagcctccagctgagcgtgtgcctgcacgaggtggcctactggtacatcctgagcatcggcgcccagaccgacttcctgagcgtgttcttcagcggctacaccttcaagcacaagatggtgtacgaggataccctgaccctgttccccttctccggcgaaaccgtgttcatgagcatggaaaaccccggcctgtggattctgggctgccacaacagcgacttcagaaaccggggcatgaccgccctgctgaaggtgtccagctgcgacaagaacaccggcgactactacgaggacagctatgaggacatcagcgcctacctgctgagcaagaacaacgccatcgagcccagatccttcagccagaacccccccgtgctgaagcggcaccagagagagatcacccggaccaccctgcagtccgaccaggaagagattgattacgacgacaccatcagcgtcgagatgaagaaagaggatttcgacatctacgacgaggacgagaaccagagcccccggtccttccagaagaaaacccggcactacttcattgccgccgtggaaagactgtgggactacggcatgagcagcagcccccacgtgctgcggaacagagcccagagcggcagcgtgccccagttcaagaaagtggtgttccaggagttcaccgacggcagcttcacccagcccctgtatcggggcgagctgaacgagcacctgggactgctgggaccttacattagagccgaggtggaagataacatcatggtcaccttcagaaaccaggcctccagaccctacagcttctacagcagcctgatcagctacgaagaggaccagcggcagggcgccgaaccccggaagaacttcgtgaagcccaacgagactaagacctacttctggaaggtgcagcaccacatggcccccacaaaggacgagttcgactgcaaggcctgggcctacttctccgatgtggacctggaaaaggacgtgcactctggcctgattggacctctgctcgtctgccacaccaacaccctgaaccccgcccacggccggcaggtcacagtgcaggaatttgccctgttcttcaccatcttcgatgagacaaagagctggtacttcaccgagaacatggaaagaaactgtagagccccctgcaacatccagatggaagatcctaccttcaaagagaactatcggttccacgccatcaacggctacatcatggacaccctgcccggcctggtcatggcccaggatcagagaatccggtggtatctgctgagcatgggcagcaacgagaacatccacagcatccacttcagcggccacgtgttcacagtgcggaagaaagaagagtacaagatggccctgtacaacctgtaccccggcgtgttcgagacagtggaaatgctgcccagcaaggccggcatctggcgggtggaatgtctgatcggcgagcatctgcacgccggaatgagcaccctgtttctggtgtacagcaacaagtgccagacccctctgggcatggccagcggccacatccgggacttccagatcaccgcctccggccagtacggccagtgggcccctaagctggcccggctccactactccggatctatcaacgcctggtccaccaaagagcccttcagctggatcaaggtggacctgctggcccctatgatcatccacggaatcaagacccagggcgccagacagaagttcagcagcctgtacatcagccagttcatcatcatgtacagcctggacggcaagaagtggcagacctaccggggcaacagcaccggcaccctgatggtgttcttcggcaacgtggacagcagcggcatcaagcacaacatcttcaacccccccatcattgcccggtacatccggctgcaccccacccactacagcatccggtccaccctgcggatggaactgatgggctgcgacctgaactcttgcagcatgcccctggggatggaaagcaaggccatcagcgacgcccagatcacagccagcagctacttcaccaacatgttcgccacctggtccccaagcaaagcccgcctgcatctccaaggcagaagcaatgcctggcggcctcaggtcaacaaccccaaagaatggctccaggtggactttcagaaaaccatgaaggtcacaggcgtgaccacccagggcgtgaaaagcctgctgacctctatgtacgtgaaagagttcctgatcagcagcagccaggacgggcaccagtggaccctgttctttcagaacggcaaagtgaaagtgttccagggcaaccaggactcctttacccccgtggtcaactctctagaccctccactgctgaccagatacctgagaatccaccctcagtcctgggtgcaccagattgccctgagaatggaagtgctgggatgcgaggcccaggatctgtactgataactcgagtcgacttaattaa

SEQ ID NO: 3 - DNA, 4371 bp, Artificial Sequence
  Parental BDD FVIII
atgcaaatagagctctccacctgcttctttctgtgccttttgcgattctgctttagtgccaccagaagatactacctgggtgcagtggaactgtcatgggactatatgcaaagtgatctcggtgagctgcctgtggacgcaagatttcctcctagagtgccaaaatcttttccattcaacacctcagtcgtgtacaaaaagactctgtttgtagaattcacggatcaccttttcaacatcgctaagccaaggccaccctggatgggtctgctaggtcctaccatccaggctgaggtttatgatacagtggtcattacacttaagaacatggcttcccatcctgtcagtcttcatgctgttggtgtatcctactggaaagcttctgagggagctgaatatgatgatcagaccagtcaaagggagaaagaagatgataaagtcttccctggtggaagccatacatatgtctggcaggtcctgaaagagaatggtccaatggcctctgacccactgtgccttacctactcatatctttctcatgtggacctggtaaaagacttgaattcaggcctcattggagccctactagtatgtagagaagggagtctggccaaggaaaagacacagaccttgcacaaatttatactactttttgctgtatttgatgaagggaaaagttggcactcagaaacaaagaactccttgatgcaggatagggatgctgcatctgctcgggcctggcctaaaatgcacacagtcaatggttatgtaaacaggtctctgccaggtctgattggatgccacaggaaatcagtctattggcatgtgattggaatgggcaccactcctgaagtgcactcaatattcctcgaaggtcacacatttcttgtgaggaaccatcgccaggcgtccttggaaatctcgccaataactttccttactgctcaaacactcttgatggaccttggacagtttctactgttttgtcatatctcttcccaccaacatgatggcatggaagcttatgtcaaagtagacagctgtccagaggaaccccaactacgaatgaaaaataatgaagaagcggaagactatgatgatgatcttactgattctgaaatggatgtggtcaggtttgatgatgacaactctccttcctttatccaaattcgctcagttgccaagaagcatcctaaaacttgggtacattacattgctgctgaagaggaggactgggactatgctcccttagtcctcgcccccgatgacagaagttataaaagtcaatatttgaacaatggccctcagcggattggtaggaagtacaaaaaagtccgatttatggcatacacagatgaaacctttaagactcgtgaagctattcagcatgaatcaggaatcttgggacctttactttatggggaagttggagacacactgttgattatatttaagaatcaagcaagcagaccatataacatctaccctcacggaatcactgatgtccgtcctttgtattcaaggagattaccaaaaggtgtaaaacatttgaaggattttccaattctgccaggagaaatattcaaatataaatggacagtgactgtagaagatgggccaactaaatcagatcctcggtgcctgacccgctattactctagtttcgttaatatggagagagatctagcttcaggactcattggccctctcctcatctgctacaaagaatctgtagatcaaagaggaaaccagataatgtcagacaagaggaatgtcatcctgttttctgtatttgatgagaaccgaagctggtacctcacagagaatatacaacgctttctccccaatccagctggagtgcagcttgaggatccagagttccaagcctccaacatcatgcacagcatcaatggctatgtttttgatagtttgcagttgtcagtttgtttgcatgaggtggcatactggtacattctaagcattggagcacagactgacttcctttctgtcttcttctctggatataccttcaaacacaaaatggtctatgaagacacactcaccctattcccattctcaggagaaactgtcttcatgtcgatggaaaacccaggtctatggattctggggtgccacaactcagactttcggaacagaggcatgaccgccttactgaaggtttctagttgtgacaagaacactggtgattattacgaggacagttatgaagatatttcagcatacttgctgagtaaaaacaatgccattgaaccaagaagcttctctcaaaacccaccagtcttgaaacgccatcaacgggaaataactcgtactactcttcagtcagatcaagaggaaattgactatgatgataccatatcagttgaaatgaagaaggaagattttgacatttatgatgaggatgaaaatcagagcccccgcagctttcaaaagaaaacacgacactattttattgctgcagtggagaggctctgggattatgggatgagtagctccccacatgttctaagaaacagggctcagagtggcagtgtccctcagttcaagaaagttgttttccaggaatttactgatggctcctttactcagcccttataccgtggagaactaaatgaacatttgggactcctggggccatatataagagcagaagttgaagataatatcatggtaactttcagaaatcaggcctctcgtccctattccttctattctagccttatttcttatgaggaagatcagaggcaaggagcagaacctagaaaaaactttgtcaagcctaatgaaaccaaaacttacttttggaaagtgcaacatcatatggcacccactaaagatgagtttgactgcaaagcctgggcttatttctctgatgttgacctggaaaaagatgtgcactcaggcctgattggaccccttctggtctgccacactaacacactgaaccctgctcatgggagacaagtgacagtacaggaatttgctctgtttttcaccatctttgatgagaccaaaagctggtacttcactgaaaatatggaaagaaactgcagggctccctgcaatatccagatggaagatcccacttttaaagagaattatcgcttccatgcaatcaatggctacataatggatacactacctggcttagtaatggctcaggatcaaaggattcgatggtatctgctcagcatgggcagcaatgaaaacatccattctattcatttcagtggacatgtgttcactgtacgaaaaaaagaggagtataaaatggcactgtacaatctctatccaggtgtttttgagacagtggaaatgttaccatccaaagctggaatttggcgggtggaatgccttattggcgagcatctacatgctgggatgagcacactttttctggtgtacagcaataagtgtcagactcccctgggaatggcttctggacacattagagattttcagattacagcttcaggacaatatggacagtgggccccaaagctggccagacttcattattccggatcaatcaatgcctggagcaccaaggagcccttttcttggatcaaggtggatctgttggcaccaatgattattcacggcatcaagacccagggtgcccgtcagaagttctccagcctctacatctctcagtttatcatcatgtatagtcttgatgggaagaagtggcagacttatcgaggaaattccactggaaccttaatggtcttctttggcaatgtggattcatctgggataaaacacaatatttttaaccctccaattattgctcgatacatccgtttgcacccaactcattatagcattcgcagcactcttcgcatggagttgatgggctgtgatttaaatagttgcagcatgccattgggaatggagagtaaagcaatatcagatgcacagattactgcttcatcctactttaccaatatgtttgccacctggtctccttcaaaagctcgacttcacctccaagggaggagtaatgcctggagacctcaggtgaataatccaaaagagtggctgcaagtggacttccagaagacaatgaaagtcacaggagtaactactcagggagtaaaatctctgcttaccagcatgtatgtgaaggagttcctcatctccagcagtcaagatggccatcagtggactctcttttttcagaatggcaaagtaaaggtttttcagggaaatcaagactccttcacacctgtggtgaactctctagacccaccgttactgactcgctaccttcgaattcacccccagagttgggtgcaccagattgccctgaggatggaggttctgggctgcgaggcacaggacctctac

SEQ ID NO: 4 - protein, 1438 aa, Artificial Sequence
  BDD FVIII
ATRRYYLGAVELSWDYMQSDLGELPVDARFPPRVPKSFPFNTSVVYKKTLFVEFTDHLFNIAKPRPPWMGLLGPTIQAEVYDTVVITLKNMASHPVSLHAVGVSYWKASEGAEYDDQTSQREKEDDKVFPGGSHTYVWQVLKENGPMASDPLCLTYSYLSHVDLVKDLNSGLIGALLVCREGSLAKEKTQTLHKFILLFAVFDEGKSWHSETKNSLMQDRDAASARAWPKMHTVNGYVNRSLPGLIGCHRKSVYWHVIGMGTTPEVHSIFLEGHTFLVRNHRQASLEISPITFLTAQTLLMDLGQFLLFCHISSHQHDGMEAYVKVDSCPEEPQLRMKNNEEAEDYDDDLTDSEMDVVRFDDDNSPSFIQIRSVAKKHPKTWVHYIAAEEEDWDYAPLVLAPDDRSYKSQYLNNGPQRIGRKYKKVRFMAYTDETFKTREAIQHESGILGPLLYGEVGDTLLIIFKNQASRPYNIYPHGITDVRPLYSRRLPKGVKHLKDFPILPGEIFKYKWTVTVEDGPTKSDPRCLTRYYSSFVNMERDLASGLIGPLLICYKESVDQRGNQIMSDKRNVILFSVFDENRSWYLTENIQRFLPNPAGVQLEDPEFQASNIMHSINGYVFDSLQLSVCLHEVAYWYILSIGAQTDFLSVFFSGYTFKHKMVYEDTLTLFPFSGETVFMSMENPGLWILGCHNSDFRNRGMTALLKVSSCDKNTGDYYEDSYEDISAYLLSKNNAIEPRSFSQNPPVLKRHQREITRTTLQSDQEEIDYDDTISVEMKKEDFDIYDEDENQSPRSFQKKTRHYFIAAVERLWDYGMSSSPHVLRNRAQSGSVPQFKKVVFQEFTDGSFTQPLYRGELNEHLGLLGPYIRAEVEDNIMVTFRNQASRPYSFYSSLISYEEDQRQGAEPRKNFVKPNETKTYFWKVQHHMAPTKDEFDCKAWAYFSDVDLEKDVHSGLIGPLLVCHTNTLNPAHGRQVTVQEFALFFTIFDETKSWYFTENMERNCRAPCNIQMEDPTFKENYRFHAINGYIMDTLPGLVMAQDQRIRWYLLSMGSNENIHSIHFSGHVFTVRKKEEYKMALYNLYPGVFETVEMLPSKAGIWRVECLIGEHLHAGMSTLFLVYSNKCQTPLGMASGHIRDFQITASGQYGQWAPKLARLHYSGSINAWSTKEPFSWIKVDLLAPMIIHGIKTQGARQKFSSLYISQFIIMYSLDGKKWQTYRGNSTGTLMVFFGNVDSSGIKHNIFNPPIIARYIRLHPTHYSIRSTLRMELMGCDLNSCSMPLGMESKAISDAQITASSYFTNMFATWSPSKARLHLQGRSNAWRPQVNNPKEWLQVDFQKTMKVTGVTTQGVKSLLTSMYVKEFLISSSQDGHQWTLFFQNGKVKVFQGNQDSFTPVVNSLDPPLLTRYLRIHPQSWVHQIALRMEVLGCEAQDLY

SEQ ID NO: 5 - DNA, 6 bp, Artificial Sequence
  MAR/ARS
atattt

SEQ ID NO: 6 - DNA, 6 bp, Artificial Sequence
  MAR/ARS
aaatat

SEQ ID NO: 7 - DNA, 6 bp, Artificial Sequence
  Potential Splice Site
ggtgat

SEQ ID NO: 8 - DNA, 5 bp, Artificial Sequence
  Destabilizing Sequence
attta

SEQ ID NO: 9 - DNA, 5 bp, Artificial Sequence
  Destabilizing Sequence
taaat

SEQ ID NO: 10 - DNA, 6 bp, Artificial Sequence
  poly-T Sequence
tttttt

SEQ ID NO: 11 - DNA, 7 bp, Artificial Sequence
  poly-A Sequence
aaaaaaa

SEQ ID NO: 12 - DNA, 5 bp, Artificial Sequence
  Promoter Binding Site
tataa

SEQ ID NO: 13 - DNA, 5 bp, Artificial Sequence
  Promoter Binding Sequence
ttata

SEQ ID NO: 14 - DNA, 8 bp, Artificial Sequence
  AU Rich Sequence Elements (ARE)
attttatt

SEQ ID NO: 15 - DNA, 8 bp, Artificial Sequence
  AU Rich Sequence Elements (ARE)
atttttaa

SEQ ID NO: 16 - DNA, 13 bp, Artificial Sequence
  Kozak Consensus Sequence
gccgccaccatgc

SEQ ID NO: 17 - protein, 32 aa, Artificial Sequence
  CTP peptide
DPRFQDSSSSKAPPPSLPSPSRLPGPSDTPIL

SEQ ID NO: 18 - protein, 28 aa, Artificial Sequence
  CTP peptide
SSSSKAPPPSLPSPSRLPGPSDTPILPQ

SEQ ID NO: 19 - protein, 11 aa, Artificial Sequence
  albumin-binding peptides core sequence
DICLPRWGCLW

SEQ ID NO: 20 - protein, 20 aa, Artificial Sequence
  PAS Sequence
ASPAAPAPASPAAPAPSAPA

SEQ ID NO: 21 - protein, 20 aa, Artificial Sequence
  PAS Sequence
AAPASPAPAAPSAPAPAAPS

SEQ ID NO: 22 - protein, 20 aa, Artificial Sequence
  PAS Sequence
APSSPSPSAPSSPSPASPSS

SEQ ID NO: 23 - protein, 19 aa, Artificial Sequence
  PAS Sequence
APSSPSPSAPSSPSPASPS

SEQ ID NO: 24 - protein, 20 aa, Artificial Sequence
  PAS Sequence
SSPSAPSPSSPASPSPSSPA

SEQ ID NO: 25 - protein, 24 aa, Artificial Sequence
  PAS Sequence
AASPAAPSAPPAAASPAAPSAPPA

SEQ ID NO: 26 - protein, 20 aa, Artificial Sequence
  PAS Sequence
ASAAAPAAASAAASAPSAAA

SEQ ID NO: 27 - DNA, 16842 bp, Homo sapiens
atgattcctgccagatttgccggggtgctgcttgctctggccctcattttgccagggaccctttgtgcagaaggaactcgcggcaggtcatccacggccctactaaggacggtctaaacggccccacgacgaacgagaccgggagtaaaacggtccctgggaaacacgtcttccttgagcgccgtccagtaggtgccggggatgcagccttttcggaagtgacttcgtcaacacctttgatgggagcatgtacagctttgcgggatactgcagttacctcctggcagggggctgccagaactacgtcggaaaagccttcactgaagcagttgtggaaactaccctcgtacatgtcgaaacgccctatgacgtcaatggaggaccgtcccccgacggtcttacgctccttctcgattattggggacttccagaatggcaagagagtgagcctctccgtgtatcttggggaattttttgacatccatttgtttgtcaatggttgcgaggaagagctaataacccctgaaggtcttaccgttctctcactcggagaggcacatagaaccccttaaaaaactgtaggtaaacaaacagttaccaaccgtgacacagggggaccaaagagtctccatgccctatgcctccaaagggctgtatctagaaactgaggctgggtactacaagctgtccggtgaggccttggcactgtgtccccctggtttctcagaggtacgggatacggaggtttcccgacatagatctttgactccgacccatgatgttcgacaggccactccggaatggctttgtggccaggatcgatggcagcggcaactttcaagtcctgctgtcagacagatacttcaacaagacctgcgggctgtgtggcaactttaacattaccgaaacaccggtcctagctaccgtcgccgttgaaagttcaggacgacagtctgtctatgaagttgttctggacgcccgacacaccgttgaaattgtactttgctgaagatgactttatgacccaagaagggaccttgacctcggacccttatgactttgccaactcatgggctctgagcagtggagaacagtggtgtgaaacgacttctactgaaatactgggttcttccctggaactggagcctgggaatactgaaacggttgagtacccgagactcgtcacctcttgtcaccacagaacgggcatctcctcccagcagctcatgcaacatctcctctggggaaatgcagaagggcctgtgggagcagtgccagcttctgaagagcacctcggtgtcttgcccgtagaggagggtcgtcgagtacgttgtagaggagacccctttacgtcttcccggacaccctcgtcacggtcgaagacttctcgtggagccacattgcccgctgccaccctctggtggaccccgagccttttgtggccctgtgtgagaagactttgtgtgagtgtgctggggggctggagtgcgcctgccctgcaacgggcgacggtgggagaccacctggggctcggaaaacaccgggacacactcttctgaaacacactcacacgaccccccgacctcacgcggacgggacgcctcctggagtacgcccggacctgtgcccaggagggaatggtgctgtacggctggaccgaccacagcgcgtgcagcccagtgtgccctgctggtatggagggaggacctcatgcgggcctggacacgggtcctcccttaccacgacatgccgacctggctggtgtcgcgcacgtcgggtcacacgggacgaccatacctctataggcagtgtgtgtccccttgcgccaggacctgccagagcctgcacatcaatgaaatgtgtcaggagcgatgcgtggatggctgcagctgccctgaggatatccgtcacacacaggggaacgcggtcctggacggtctcggacgtgtagttactttacacagtcctcgctacgcacctaccgacgtcgacgggactccgacagctcctggatgaaggcctctgcgtggagagcaccgagtgtccctgcgtgcattccggaaagcgctaccctcccggcacctccctctctcgagactgctgtcgaggacctacttccggagacgcacctctcgtggctcacagggacgcacgtaaggcctttcgcgatgggagggccgtggagggagagagctctgaccaacacctgcatttgccgaaacagccagtggatctgcagcaatgaagaatgtccaggggagtgccttgtcactggtcaatcccacttcaagagctttgacgttgtggacgtaaacggctttgtcggtcacctagacgtcgttacttcttacaggtcccctcacggaacagtgaccagttagggtgaagttctcgaaactgaacagatacttcaccttcagtgggatctgccagtacctgctggcccgggattgccaggaccactccttctccattgtcattgagactgtccagtgtgctgttgtctatgaagtggaagtcaccctagacggtcatggacgaccgggccctaacggtcctggtgaggaagaggtaacagtaactctgacaggtcacacgacatgaccgcgacgctgtgtgcacccgctccgtcaccgtccggctgcctggcctgcacaacagccttgtgaaactgaagcatggggcaggagttgccatggatactggcgctgcgacacacgtgggcgaggcagtggcaggccgacggaccggacgtgttgtcggaacactttgacttcgtaccccgtcctcaacggtaccttggccaggacatccagctccccctcctgaaaggtgacctccgcatccagcatacagtgacggcctccgtgcgcctcagctacggggaggacctgcagatgaccggtcctgtaggtcgagggggaggactttccactggaggcgtaggtcgtatgtcactgccggaggcacgcggagtcgatgcccctcctggacgtctacgactgggatggccgcgggaggctgctggtgaagctgtcccccgtctatgccgggaagacctgcggcctgtgtgggaattacaatggcaaccagggcgacgctgaccctaccggcgccctccgacgaccacttcgacagggggcagatacggcccttctggacgccggacacacccttaatgttaccgttggtcccgctgcacttccttaccccctctgggctggcrgagccccgggtggaggacttcgggaacgcctggaagctgcacggggactgccaggacctgcagaagcagcacagtgaaggaatgggggagacccgaccgyctcggggcccacctcctgaagcccttgcggaccttcgacgtgcccctgacggtcctggacgtcttcgtcgtgtccgatccctgcgccctcaacccgcgcatgaccaggttctccgaggaggcgtgcgcggtcctgacgtcccccacattcgaggcctgccatcgtgccgtcagcgctagggacgcgggagttgggcgcgtactggtccaagaggctcctccgcacgcgccaggactgcagggggtgtaagctccggacggtagcacggcagtcgccgctgccctacctgcggaactgccgctacgacgtgtgctcctgctcggacggccgcgagtgcctgtgcggcgccctggccagctatgccgcggcctgcgggcgacgggatggacgccttgacggcgatgctgcacacgaggacgagcctgccggcgctcacggacacgccgcgggaccggtcgatacggcgccggacgccggggagaggcgtgcgcgtcgcgtggcgcgagccaggccgctgtgagctgaactgcccgaaaggccaggtgtacctgcagtgcgggaccccctgcaacctgcccctctccgcacgcgcagcgcaccgcgctcggtccggcgacactcgacttgacgggctttccggtccacatggacgtcacgccctgggggacgttggagacctgccgctctctctcttacccggatgaggaatgcaatgaggcctgcctggagggctgcttctgccccccagggctctacatggatgagaggggggacctggacggcgagagagagaatgggcctactccttacgttactccggacggacctcccgacgaagacggggggtcccgagatgtacctactctcccccctgtgcgtgcccaaggcccagtgcccctgttactatgacggtgagatcttccagccagaagacatcttctcagaccatcacaccatgtgctactgtgaggatgacgcacgggttccgggtcacggggacaatgatactgccactctagaaggtcggtcttctgtagaagagtctggtagtgtggtacacgatgacactcctacgcttcatgcactgtaccatgagtggagtccccggaagcttgctgcctgacgctgtcctcagcagtcccctgtctcatcgcagcaaaaggagcctatcctgcgaagtacgtgacatggtactcacctcaggggccttcgaacgacggactgcgacaggagtcgtcaggggacagagtagcgtcgttttcctcggataggactcggccccccatggtcaagctggtgtgtcccgctgacaacctgcgggctgaagggctcgagtgtaccaaaacgtgccagaactatgacctggagtgcatgagccggggggtaccagttcgaccacacagggcgactgttggacgcccgacttcccgagctcacatggttttgcacggtcttgatactggacctcacgtacagcatgggctgtgtctctggctgcctctgccccccgggcatggtccggcatgagaacagatgtgtggccctggaaaggtgtccctgcttccatcagggcatcgtacccgacacagagaccgacggagacggggggcccgtaccaggccgtactcttgtctacacaccgggacctttccacagggacgaaggtagtcccgtaggagtatgcccctggagaaacagtgaagattggctgcaacacttgtgtctgtcgggaccggaagtggaactgcacagaccatgtgtgtgatgccacgtgtcctcatacggggacctctttgtcacttctaaccgacgttgtgaacacagacagccctggccttcaccttgacgtgtctggtacacacactacggtgcacctccacgatcggcatggcccactacctcaccttcgacgggctcaaatacctgttccccggggagtgccagtacgttctggtgcaggattactgcggcagtgaggtgctagccgtaccgggtgatggagtggaagctgcccgagtttatggacaaggggcccctcacggtcatgcaagaccacgtcctaatgacgccgtcaaaccctgggacctttcggatcctagtggggaataagggatgcagccacccctcagtgaaatgcaagaaacgggtcaccatcctggtggagggaggagagattgggaccctggaaagcctaggatcaccccttattccctacgtcggtggggagtcactttacgttctttgcccagtggtaggaccacctccctcctctctttgagctgtttgacggggaggtgaatgtgaagaggcccatgaaggatgagactcactttgaggtggtggagtctggccggtacatcattctgctgctgggaactcgacaaactgcccctccacttacacttctccgggtacttcctactctgagtgaaactccaccacctcagaccggccatgtagtaagacgacgaccccaaagccctctccgtggtctgggaccgccacctgagcatctccgtggtcctgaagcagacataccaggagaaagtgtgtggcctgtgtgggaattttgatgtttcgggagaggcaccagaccctggcggtggactcgtagaggcaccaggacttcgtctgtatggtcctctttcacacaccggacacacccttaaaactaggcatccagaacaatgacctcaccagcagcaacctccaagtggaggaagaccctgtggactttgggaactcctggaaagtgagctcgcagtgtgctgacaccgtaggtcttgttactggagtggtcgtcgttggaggttcacctccttctgggacacctgaaacccttgaggacctttcactcgagcgtcacacgactgtccagaaaagtgcctctggactcatcccctgccacctgccataacaacatcatgaagcagacgatggtggattcctcctgtagaatccttaccagtgacgtggtcttttcacggagacctgagtaggggacggtggacggtattgttgtagtacttcgtctgctaccacctaaggaggacatcttaggaatggtcactgcacttccaggactgcaacaagctggtggaccccgagccatatctggatgtctgcatttacgacacctgctcctgtgagtccattggggactgcgcctgcttcgaaggtcctgacgttgttcgaccacctggggctcggtatagacctacagacgtaaatgctgtggacgaggacactcaggtaacccctgacgcggacgaagtgcgacaccattgctgcctatgcccacgtgtgtgcccagcatggcaaggtggtgacctggaggacggccacattgtgcccccagagctgcgaggagaggaacgctgtggtaacgacggatacgggtgcacacacgggtcgtaccgttccaccactggacctcctgccggtgtaacacgggggtctcgacgctcctctcctatctccgggagaacgggtatgagtgtgagtggcgctataacagctgtgcacctgcctgtcaagtcacgtgtcagcaccctgagccactggcctgccctgttagaggccctcttgcccatactcacactcaccgcgatattgtcgacacgtggacggacagttcagtgcacagtcgtgggactcggtgaccggacgggacagcagtgtgtggagggctgccatgcccactgccctccagggaaaatcctggatgagcttttgcagacctgcgttgaccctgaagactgtccagtgtgtgagcgtcacacacctcccgacggtacgggtgacgggaggtcccttttaggacctactcgaaaacgtctggacgcaactgggacttctgacaggtcacacactcgtggctggccggcgttttgcctcaggaaagaaagtcaccttgaatcccagtgaccctgagcactgccagatttgccactgtgatgttgtcaacctcacctcaccgaccggccgcaaaacggagtcctttctttcagtggaacttagggtcactgggactcgtgacggtctaaacggtgacactacaacagttggagtggagtgaagcctgccaggagccgggaggcctggtggtgcctcccacagatgccccggtgagccccaccactctgtatgtggaggacatctcggaaccgccgttcacttcggacggtcctcggccctccggaccaccacggagggtgtctacggggccactcggggtggtgagacatacacctcctgtagagccttggcggcaagcacgatttctactgcagcaggctactggacctggtcttcctgctggatggctcctccaggctgtccgaggctgagtttgaagtgctgaaggcctttgtgcgtgctaaagatgacgtcgtccgatgacctggaccagaaggacgacctaccgaggaggtccgacaggctccgactcaaacttcacgacttccggaaacacgtggacatgatggagcggctgcgcatctcccagaagtgggtccgcgtggccgtggtggagtaccacgacggctcccacgcctacatcgggctcaaggacccacctgtactacctcgccgacgcgtagagggtcttcacccaggcgcaccggcaccacctcatggtgctgccgagggtgcggatgtagcccgagttcctggggaagcgaccgtcagagctgcggcgcattgccagccaggtgaagtatgcgggcagccaggtggcctccaccagcgaggtcttgaaatacacactgttccaccttcgctggcagtctcgacgccgcgtaacggtcggtccacttcatacgcccgtcggtccaccggaggtggtcgctccagaactttatgtgtgacaaggtaatcttcagcaagatcgaccgccctgaagcctcccgcatcgccctgctcctgatggccagccaggagccccaacggatgtcccggaactttgtccgctacttagaagtcgttctagctggcgggacttcggagggcgtagcgggacgaggactaccggtcggtcctcggggttgcctacagggccttgaaacaggcgatggtccagggcctgaagaagaagaaggtcattgtgatcccggtgggcattgggccccatgccaacctcaagcagatccgcctcatcgagaagcaggcccctgcaggtcccggacttcttcttcttccagtaacactagggccacccgtaacccggggtacggttggagttcgtctaggcggagtagctcttcgtccggggacagaacaaggccttcgtgctgagcagtgtggatgagctggagcagcaaagggacgagatcgttagctacctctgtgaccttgcccctgaagcccctcctcctcttgttccggaagcacgactcgtcacacctactcgacctcgtcgtttccctgctctagcaatcgatggagacactggaacggggacttcggggaggaggtactctgccccccgacatggcacaagtcactgtgggcccggggctcttgggggtttcgaccctggggcccaagaggaactccatggttctggatgtggcgatgagacggggggctgtaccgtgttcagtgacacccgggccccgagaacccccaaagctgggaccccgggttctccttgaggtaccaagacctacaccgcttcgtcctggaaggatcggacaaaattggtgaagccgacttcaacaggagcaaggagttcatggaggaggtgattcagcggatggatgtgggccaggacaaagcaggaccttcctagcctgttttaaccacttcggctgaagttgtcctcgttcctcaagtacctcctccactaagtcgcctacctacacccggtcctgtgcatccacgtcacggtgctgcagtactcctacatggtgaccgtggagtaccccttcagcgaggcacagtccaaaggggacatcctgcagcgggtgcgagacgtaggtgcagtgccacgacgtcatgaggatgtaccactggcacctcatggggaagtcgctccgtgtcaggtttcccctgtaggacgtcgcccacgctctgatccgctaccagggcggcaacaggaccaacactgggctggccctgcggtacctctctgaccacagcttcttggtcagccagggtgaccgggagcaggcgctaggcgatggtcccgccgttgtcctggttgtgacccgaccgggacgccatggagagactggtgtcgaagaaccagtcggtcccactggccctcgtccgccccaacctggtctacatggtcaccggaaatcctgcctctgatgagatcaagaggctgcctggagacatccaggtggtgcccattggagtgggccctaatggggttggaccagatgtaccagtggcctttaggacggagactactctagttctccgacggacctctgtaggtccaccacgggtaacctcacccgggattacccaacgtgcaggagctggagaggattggctggcccaatgcccctatcctcatccaggactttgagacgctcccccgagaggctcctgacctggtgctgcaggttgcacgtcctcgacctctcctaaccgaccgggttacggggataggagtaggtcctgaaactctgcgagggggctctccgaggactggaccacgacgtgaggtgctgctccggagaggggctgcagatccccaccctctcccctgcacctgactgcagccagcccctggacgtgatccttctcctggatggctcctccctccacgacgaggcctctccccgacgtctaggggtgggagaggggacgtggactgacgtcggtcggggacctgcactaggaagaggacctaccgaggaggagtttcccagcttcttattttgatgaaatgaagagtttcgccaaggctttcatttcaaaagccaatatagggcctcgtctcactcaggtgtcagtgctgctcaaagggtcgaagaataaaactactttacttctcaaagcggttccgaaagtaaagttttcggttatatcccggagcagagtgagtccacagtcacgacgagtatggaagcatcaccaccattgacgtgccatggaacgtggtcccggagaaagcccatttgctgagccttgtggacgtcatgcagcgggagggaggccctcataccttcgtagtggtggtaactgcacggtaccttgcaccagggcctctttcgggtaaacgactcggaacacctgcagtacgtcgccctccctccgggcagccaaatcggggatgccttgggctttgctgtgcgatacttgacttcagaaatgcatggtgccaggccgggagcctcaaaggcggtggtcatcctggtcgtcggtttagcccctacggaacccgaaacgacacgctatgaactgaagtctttacgtaccacggtccggccctcggagtttccgccaccagtaggaccagacggacgtctctgtggattcagtggatgcagcagctgatgccgccaggtccaacagagtgacagtgttccctattggaattggagatcgctacgatgcagtgcctgcagagacacctaagtcacctacgtcgtcgactacggcggtccaggttgtctcactgtcacaagggataaccttaacctctagcgatgctacgtccccagctacggatcttggcaggcccagcaggcgactccaacgtggtgaagctccagcgaatcgaagacctccctaccatggtcaccttgggcaattccttgggtcgatgcctagaaccgtccgggtcgtccgctgaggttgcaccacttcgaggtcgcttagcttctggagggatggtaccagtggaacccgttaaggaacctccacaaactgtgctctggatttgttaggatttgcatggatgaggatgggaatgagaagaggcccggggacgtctggaccttgccagaccagtgccacggaggtgtttgacacgagacctaaacaatcctaaacgtacctactcctacccttactcttctccgggcccctgcagacctggaacggtctggtcacggtgaccgtgacttgccagccagatggccagaccttgctgaagagtcatcgggtcaactgtgaccgggggctgaggccttcgtgccctaacagccagtcccctgtggcactgaacggtcggtctaccggtctggaacgacttctcagtagcccagttgacactggcccccgactccggaagcacgggattgtcggtcaggggacttaaagtggaagagacctgtggctgccgctggacctgcccctgygtgtgcacaggcagctccactcggcacatcgtgacctttgatgggcagaatttcaaaatttcaccttctctggacaccgacggcgacctggacggggacrcacacgtgtccgtcgaggtgagccgtgtagcactggaaactacccgtcttaaagttgctgactggcagctgttcttatgtcctatttcaaaacaaggagcaggacctggaggtgattctccataatggtgcctgcagccctggagcaaggcagggccgactgaccgtcgacaagaatacaggataaagttttgttcctcgtcctggacctccactaagaggtattaccacggacgtcgggacctcgttccgtcccgtgcatgaaatccatcgaggtgaagcacagtgccctctccgtcgagstgcacagtgacatggaggtgacggtgaatgggagactggtctctgttccttacgacgtactttaggtagctccacttcgtgtcacgggagaggcagctcsacgtgtcactgtacctccactgccacttaccctctgaccagagacaaggaatgctgggtgggaacatggaagtcaacgtttatggtgccatcatgcatgaggtcagattcaatcaccttggtcacatcttcacattcactccacaaaacaatgaacccacccttgtaccttcagttgcaaataccacggtagtacgtactccagtctaagttagtggaaccagtgtagaagtgtaagtgaggtgttttgttactgttccaactgcagctcagccccaagacttttgcttcaaagacgtatggtctgtgtgggatctgtgatgagaacggagccaatgacttcatgctgagggatcaaggttgacgtcgagtcggggttctgaaaacgaagtttctgcataccagacacaccctagacactactcttgcctcggttactgaagtacgactccctaggcacagtcaccacagactggaaaacacttgttcaggaatggactgtgcagcggccagggcagacgtgccagcccatcctggaggagcagtgtcttgtccccgtgtcagtggtgtctgaccttttgtgaacaagtccttacctgacacgtcgccggtcccgtctgcacggtcgggtaggacctcctcgtcacagaacaggccgacagctcccactgccaggtcctcctcttaccactgtttgctgaatgccacaaggtcctggctccagccacattctatgccatctgccagcaggacagggctgtcgagggtgacggtccaggaggagaatggtgacaaacgacttacggtgttccaggaccgaggtcggtgtaagatacggtagacggtcgtcctgtcttgccaccaggagcaagtgtgtgaggtgatcgcctcttatgcccacctctgtcggaccaacggggtctgcgttgactggaggacacctgatttctgtgctaacggtggtcctcgttcacacactccactagcggagaatacgggtggagacagcctggttgccccagacgcaactgacctcctgtggactaaagacacgaatgtcatgcccaccatctctggtctacaaccactgtgagcatggctgtccccggcactgtgatggcaacgtgagctcctgtggggaccatccctccgaagtacagtacgggtggtagagaccagatgttggtgacactcgtaccgacaggggccgtgacactaccgttgcactcgaggacacccctggtagggaggcttcgctgtttctgccctccagataaagtcatgttggaaggcagctgtgtccctgaagaggcctgcactcagtgcattggtgaggatggagtccagcaccagttcgacaaagacgggaggtctatttcagtacaaccttccgtcgacacagggacttctccggacgtgagtcacgtaaccactcctacctcaggtcgtggtcaacctggaagcctgggtcccggaccaccagccctgtcagatctgcacatgcctcagcgggcggaaggtcaactgcacaacgcagccctgccccacggccaaaggaccttcggacccagggcctggtggtcgggacagtctagacgtgtacggagtcgcccgccttccagttgacgtgttgcgtcgggacggggtgccggtttgctcccacgtgtggcctgtgtgaagtagcccgcctccgccagaatgcagaccagtgctgccccgagtatgagtgtgtgtgtgacccagtgagctgtgacccgagggtgcacaccggacacacttcatcgggcggaggcggtcttacgtctggtcacgacggggctcatactcacacacacactgggtcactcgacactggtgcccccagtgcctcactgtgaacgtggcctccagcccacactgaccaaccctggcgagtgcagacccaacttcacctgcgcctgcaggaaggaggagtgacgggggtcacggagtgacacttgcaccggaggtcgggtgtgactggttgggaccgctcacgtctgggttgaagtggacgcggacgtccttcctcctcaccaaaagagtgtccccaccctcctgccccccgcaccgtttgcccacccttcggaagacccagtgctgtgatgagtatgagtgtgcctgcaactgtgtcaacgttttctcacaggggtgggaggacggggggcgtggcaaacgggtgggaagccttctgggtcacgacactactcatactcacacggacgttgacacagttgtccacagtgagctgtccccttgggtacttggcctcaaccgccaccaatgactgtggctgtaccacaaccacctgccttcccgacaaggtgtgtgtccaccaggtgtcactcgacaggggaacccatgaaccggagttggcggtggttactgacaccgacatggtgttggtggacggaagggctgttccacacacaggtgggaagcaccatctaccctgtgggccagttctgggaggagggctgcgatgtgtgcacctgcaccgacatggaggatgccgtgatgggcctccgcgtggcccacttcgtggtagatgggacacccggtcaagaccctcctcccgacgctacacacgtggacgtggctgtacctcctacggcactacccggaggcgcaccgggtgtgctcccagaagccctgtgaggacagctgtcggtcgggcttcacttacgttctgcatgaaggcgagtgctgtggaaggtgcctgccatctgcctgtgagcacgagggtcttcgggacactcctgtcgacagccagcccgaagtgaatgcaagacgtacttccgctcacgacaccttccacggacggtagacggacactcgtggtgactggctcaccgcggggggactcccagtcttcctggaagagtgtcggctcccagtgggcctccccggagaacccctgcctcatcaatgagtgtgcaccactgaccgagtggcgcccccctgagggtcagaaggaccttctcacagccgagggtcacccggaggggcctcttggggacggagtagttactcacactccgagtgaaggaggaggtctttatacaacaaaggaacgtctcctgcccccagctggaggtccctgtctgcccctcgggctttcagctgagctgtaagacaggctcacttcctcctccagaaatatgttgtttccttgcagaggacgggggtcgacctccagggacagacggggagcccgaaagtcgactcgacattctgctcagcgtgctgcccaagctgtcgctgtgagcgcatggaggcctgcatgctcaatggcactgtcattgggcccgggaagactgtgatgatcgatgtgtgcgagtcgcacgacgggttcgacagcgacactcgcgtacctccggacgtacgagttaccgtgacagtaacccgggcccttctgacactactagctacacacgacgacctgccgctgcatggtgcaggtgggggtcatctctggattcaagctggagtgcaggaagaccacctgcaacccctgccccctgggttacaaggaagtgctggacggcgacgtaccacgtccacccccagtagagacctaagttcgacctcacgtccttctggtggacgttggggacgggggacccaatgttccttcaaaataacacaggtgaatgttgtgggagatgtttgcctacggcttgcaccattcagctaagaggaggacagatcatgacactgaagcgtgatgagacgctttttattgtgtccacttacaacaccctctacaaacggatgccgaacgtggtaagtcgattctcctcctgtctagtactgtgacttcgcactactctgcgaccaggatggctgtgatactcacttctgcaaggtcaatgagagaggagagtacttctgggagaagagggtcacaggctgcccaccctttgatgaacacaagggtcctaccgacactatgagtgaagacgttccagttactctctcctctcatgaagaccctcttctcccagtgtccgacgggtgggaaactacttgtgttctgtcttgctgagggaggtaaaattatgaaaattccaggcacctgctgtgacacatgtgaggagcctgagtgcaacgacatcactgccaggctgcagtatgacagaacgactccctccattttaatacttttaaggtccgtggacgacactgtgtacactcctcggactcacgttgctgtagtgacggtccgacgtcatactcaaggtgggaagctgtaagtctgaagtagaggtggatatccactactgccagggcaaatgtgccagcaaagccatgtactccattgacatcaacgatgtagttccacccttcgacattcagacttcatctccacctataggtgatgacggtcccgtttacacggtcgtttcggtacatgaggtaactgtagttgctacagcaggaccagtgctcctgctgctctccgacacggacggagcccatgcaggtggccctgcactgcaccaatggctctgttgtgtaccatgaggttctcaatcgtcctggtcacgaggacgacgagaggctgtgcctgcctcgggtacgtccaccgggacgtgacgtggttaccgagacaacacatggtactccaagagttagccatggagtgcaaatgctcccccaggaagtgcagcaagtga

SEQ ID NO: 28 - protein, 2813 aa, Homo sapiens
  variant (2016)..(2016): Xaa can be any naturally occurring amino acid
MIPARFAGVLLALALILPGTLCAEGTRGRSSTARCSLFGSDFVNTFDGSMYSFAGYCSYLLAGGCQKRSFSIIGDFQNGKRVSLSVYLGEFFDIHLFVNGTVTQGDQRVSMPYASKGLYLETEAGYYKLSGEAYGFVARIDGSGNFQVLLSDRYFNKTCGLCGNFNIFAEDDFMTQEGTLTSDPYDFANSWALSSGEQWCERASPPSSSCNISSGEMQKGLWEQCQLLKSTSVFARCHPLVDPEPFVALCEKTLCECAGGLECACPALLEYARTCAQEGMVLYGWTDHSACSPVCPAGMEYRQCVSPCARTCQSLHINEMCQERCVDGCSCPEGQLLDEGLCVESTECPCVHSGKRYPPGTSLSRDCNTCICRNSQWICSNEECPGECLVTGQSHFKSFDNRYFTFSGICQYLLARDCQDHSFSIVIETVQCADDRDAVCTRSVTVRLPGLHNSLVKLKHGAGVAMDGQDIQLPLLKGDLRIQHTVTASVRLSYGEDLQMDWDGRGRLLVKLSPVYAGKTCGLCGNYNGNQGDDFLTPSGLAEPRVEDFGNAWKLHGDCQDLQKQHSDPCALNPRMTRFSEEACAVLTSPTFEACHRAVSPLPYLRNCRYDVCSCSDGRECLCGALASYAAACAGRGVRVAWREPGRCELNCPKGQVYLQCGTPCNLTCRSLSYPDEECNEACLEGCFCPPGLYMDERGDCVPKAQCPCYYDGEIFQPEDIFSDHHTMCYCEDGFMHCTMSGVPGSLLPDAVLSSPLSHRSKRSLSCRPPMVKLVCPADNLRAEGLECTKTCQNYDLECMSMGCVSGCLCPPGMVRHENRCVALERCPCFHQGKEYAPGETVKIGCNTCVCRDRKWNCTDHVCDATCSTIGMAHYLTFDGLKYLFPGECQYVLVQDYCGSNPGTFRILVGNKGCSHPSVKCKKRVTILVEGGEIELFDGEVNVKRPMKDETHFEVVESGRYIILLLGKALSVVWDRHLSISVVLKQTYQEKVCGLCGNFDGIQNNDLTSSNLQVEEDPVDFGNSWKVSSQCADTRKVPLDSSPATCHNNIMKQTMVDSSCRILTSDVFQDCNKLVDPEPYLDVCIYDTCSCESIGDCACFCDTIAAYAHVCAQHGKVVTWRTATLCPQSCEERNLRENGYECEWRYNSCAPACQVTCQHPEPLACPVQCVEGCHAHCPPGKILDELLQTCVDPEDCPVCEVAGRRFASGKKVTLNPSDPEHCQICHCDVVNLTCEACQEPGGLVVPPTDAPVSPTTLYVEDISEPPLHDFYCSRLLDLVFLLDGSSRLSEAEFEVLKAFVVDMMERLRISQKWVRVAVVEYHDGSHAYIGLKDRKRPSELRRIASQVKYAGSQVASTSEVLKYTLFQIFSKIDRPEASRIALLLMASQEPQRMSRNFVRYVQGLKKKKVIVIPVGIGPHANLKQIRLIEKQAPENKAFVLSSVDELEQQRDEIVSYLCDLAPEAPPPTLPPDMAQVTVGPGLLGVSTLGPKRNSMVLDVAFVLEGSDKIGEADFNRSKEFMEEVIQRMDVGQDSIHVTVLQYSYMVTVEYPFSEAQSKGDILQRVREIRYQGGNRTNTGLALRYLSDHSFLVSQGDREQAPNLVYMVTGNPASDEIKRLPGDIQVVPIGVGPNANVQELERIGWPNAPILIQDFETLPREAPDLVLQRCCSGEGLQIPTLSPAPDCSQPLDVILLLDGSSSFPASYFDEMKSFAKAFISKANIGPRLTQVSVLQYGSITTIDVPWNVVPEKAHLLSLVDVMQREGGPSQIGDALGFAVRYLTSEMHGARPGASKAVVILVTDVSVDSVDAAADAARSNRVTVFPIGIGDRYDAAQLRILAGPAGDSNVVKLQRIEDLPTMVTLGNSFLHKLCSGFVRICMDEDGNEKRPGDVWTLPDQCHTVTCQPDGQTLLKSHRVNCDRGLRPSCPNSQSPVKVEETCGCRWTCPCVCTGSSTRHIVTFDGQNFKLTGSCSYVLFQNKEQDLEVILHNGACSPGARQGCMKSIEVKHSALSVEXHSDMEVTVNGRLVSVPYVGGNMEVNVYGAIMHEVRFNHLGHIFTFTPQNNEFQLQLSPKTFASKTYGLCGICDENGANDFMLRDGTVTTDWKTLVQEWTVQRPGQTCQPILEEQCLVPDSSHCQVLLLPLFAECHKVLAPATFYAICQQDSCHQEQVCEVIASYAHLCRTNGVCVDWRTPDFCAMSCPPSLVYNHCEHGCPRHCDGNVSSCGDHPSEGCFCPPDKVMLEGSCVPEEACTQCIGEDGVQHQFLEAWVPDHQPCQICTCLSGRKVNCTTQPCPTAKAPTCGLCEVARLRQNADQCCPEYECVCDPVSCDLPPVPHCERGLQPTLTNPGECRPNFTCACRKEECKRVSPPSCPPHRLPTLRKTQCCDEYECACNCVNSTVSCPLGYLASTATNDCGCTTTTCLPDKVCVHRSTIYPVGQFWEEGCDVCTCTDMEDAVMGLRVAQCSQKPCEDSCRSGFTYVLHEGECCGRCLPSACEVVTGSPRGDSQSSWKSVGSQWASPENPCLINECVRVKEEVFIQQRNVSCPQLEVPVCPSGFQLSCKTSACCPSCRCERMEACMLNGTVIGPGKTVMIDVCTTCRCMVQVGVISGFKLECRKTTCNPCPLGYKEENNTGECCGRCLPTACTIQLRGGQIMTLKRDETLQDGCDTHFCKVNERGEYFWEKRVTGCPPFDEHKCLAEGGKIMKIPGTCCDTCEEPECNDITARLQYVKVGSCKSEVEVDIHYCQGKCASKAMYSIDINDVQDQCSCCSPTRTEPMQVALHCTNGSVVYHEVLNAMECKCSPRKCSK

SEQ ID NO: 29 - protein, 4 aa, Artificial Sequence
  human IgG1
ELLG

SEQ ID NO: 30 - protein, 42 aa, Artificial Sequence
  XTEN AE42-4
GAPGSPAGSPTSTEEGTSESATPESGPGSEPATSGSETPASS

SEQ ID NO: 31 - DNA, 126 bp, Artificial Sequence
  XTEN AE42-4
ggcgcgccaggttctcctgctggctcccccacctcaacagaagaggggacaagcgaaagcgctacgcctgagagtggccctggctctgagccagccacctccggctctgaaacccctgcctcgagc

SEQ ID NO: 32 - protein, 144 aa, Artificial Sequence
  XTEN AE144-2A
TSTEPSEGSAPGSPAGSPTSTEEGTSTEPSEGSAPGTSTEPSEGSAPGTSESATPESGPGTSTEPSEGSAPGTSESATPESGPGSEPATSGSETPGTSTEPSEGSAPGTSTEPSEGSAPGTSESATPESGPGTSESATPESGPG

SEQ ID NO: 33 - DNA, 450 bp, Artificial Sequence
  XTEN AE144-2A
ggcgcgccaaccagtacggagccgtccgaggggagcgcaccaggaagcccggctgggagcccgacttctaccgaagagggtacatctaccgaaccaagtgaaggttcagcaccaggcacctcaacagaaccctctgagggctcggcgcctggtacaagtgagtccgccaccccagaatccgggcctgggacaagcacagaaccttcggaagggagtgcccctggaacatccgaatcggcaaccccagaatcagggccaggatctgagcccgcgacttcgggctccgagacgcctgggacatccaccgagccctccgaaggatcagccccaggcaccagcacggagccctctgagggaagcgcacctggtaccagcgaaagcgcaactcccgaatcaggtcccggtacgagcgagtcggcgaccccggagagcgggccaggtgcctcgagc

SEQ ID NO: 34 - protein, 144 aa, Artificial Sequence
  XTEN AE144-3B
SPAGSPTSTEEGTSESATPESGPGSEPATSGSETPGTSESATPESGPGTSTEPSEGSAPGTSTEPSEGSAPGTSTEPSEGSAPGTSTEPSEGSAPGTSTEPSEGSAPGTSTEPSEGSAPGSPAGSPTSTEEGTSTEPSEGSAPG

SEQ ID NO: 35 - DNA, 450 bp, Artificial Sequence
  XTEN AE144-3B
ggcgcgccaagtcccgctggaagcccaactagcaccgaagaggggacctcagagtccgccacccccgagtccggccctggctctgagcctgccactagcggctccgagactcctggcacatccgaaagcgctacacccgagagtggacccggcacctctaccgagcccagtgagggctccgcccctggaacaagcaccgagcccagcgaaggcagcgccccagggacctccacagagcccagtgaaggcagtgctcctggcaccagcaccgaaccaagcgagggctctgcacccgggacctccaccgagccaagcgaaggctctgcccctggcacttccaccgagcccagcgaaggcagcgcccctgggagccccgctggctctcccaccagcactgaggagggcacatctaccgaaccaagtgaaggctctgcaccaggtgcctcgagc

SEQ ID NO: 36 - protein, 144 aa, Artificial Sequence
  XTEN AE144-4A
TSESATPESGPGSEPATSGSETPGTSESATPESGPGSEPATSGSETPGTSESATPESGPGTSTEPSEGSAPGTSESATPESGPGSPAGSPTSTEEGSPAGSPTSTEEGSPAGSPTSTEEGTSESATPESGPGTSTEPSEGSAPG

SEQ ID NO: 37 - DNA, 450 bp, Artificial Sequence
  XTEN AE144-4A
ggcgcgccaacgtccgaaagtgctacccctgagtcaggccctggtagtgagcctgccacaagcggaagcgaaactccggggacctcagagtctgccactcccgaatcggggccaggctctgaaccggccacttcagggagcgaaacaccaggaacatcggagagcgctaccccggagagcgggccaggaactagtactgagcctagcgagggaagtgcacctggtacaagcgagtccgccacacccgagtctggccctggctctccagcgggctcacccacgagcactgaagagggctctcccgctggcagcccaacgtcgacagaagaaggatcaccagcaggctcccccacatcaacagaggagggtacatcagaatctgctactcccgagagtggacccggtacctccactgagcccagcgaggggagtgcaccaggtgcctcgagc

SEQ ID NO: 38 - protein, 144 aa, Artificial Sequence
  XTEN AE144-5A
TSESATPESGPGSEPATSGSETPGTSESATPESGPGSEPATSGSETPGTSESATPESGPGTSTEPSEGSAPGSPAGSPTSTEEGTSESATPESGPGSEPATSGSETPGTSESATPESGPGSPAGSPTSTEEGSPAGSPTSTEEG

SEQ ID NO: 39 - DNA, 450 bp, Artificial Sequence
  XTEN AE144-5A
ggcgcgccaacatcagagagcgccacccctgaaagtggtcccgggagcgagccagccacatctgggtcggaaacgccaggcacaagtgagtctgcaactcccgagtccggacctggctccgagcctgccactagcggctccgagactccgggaacttccgagagcgctacaccagaaagcggacccggaaccagtaccgaacctagcgagggctctgctccgggcagcccagccggctctcctacatccacggaggagggcacttccgaatccgccaccccggagtcagggccaggatctgaacccgctacctcaggcagtgagacgccaggaacgagcgagtccgctacaccggagagtgggccagggagccctgctggatctcctacgtccactgaggaagggtcaccagcgggctcgcccaccagcactgaagaaggtgcctcgagc

SEQ ID NO: 40 - protein, 144 aa, Artificial Sequence
  XTEN AE144-6B
TSTEPSEGSAPGTSESATPESGPGTSESATPESGPGTSESATPESGPGSEPATSGSETPGSEPATSGSETPGSPAGSPTSTEEGTSTEPSEGSAPGTSTEPSEGSAPGSEPATSGSETPGTSESATPESGPGTSTEPSEGSAPG

SEQ ID NO: 41 - DNA, 450 bp, Artificial Sequence
  XTEN AE144-6B
ggcgcgccaacatctaccgagccttccgaaggctctgcccctgggacctcagaatctgcaacccctgaaagcggccctggaacctccgaaagtgccactcccgagagcggcccagggacaagcgagtcagcaacccctgagtctggacccggcagcgagcctgcaacctctggctcagagactcccggctcagaacccgctacctcaggctccgagacacccggctctcctgctgggagtcccacttccaccgaggaaggaacatccactgagcctagtgagggctctgcccctggaaccagcacagagccaagtgagggcagtgcaccaggatccgagccagcaaccagcgggtccgagactcccgggacctctgagtctgccaccccagagagcggacccggcacttcaaccgagccctccgaaggatcagcaccaggtgcctcgagc

SEQ ID NO: 42 - protein, 144 aa, Artificial Sequence
  XTEN AG144-1
PGSSPSASTGTGPGSSPSASTGTGPGTPGSGTASSSPGSSTPSGATGSPGSSPSASTGTGPGASPGTSSTGSPGTPGSGTASSSPGSSTPSGATGSPGTPGSGTASSSPGASPGTSSTGSPGASPGTSSTGSPGTPGSGTASSS

SEQ ID NO: 43 - DNA, 450 bp, Artificial Sequence
  XTEN AG144-1
ggcgcgccacccgggtcgtccccgtcggcgtccaccggaacagggccagggtcatccccgtcagcgtcgactgggacgggacccgggacacccggttcggggactgcatcctcctcgcctggttcgtccaccccgtcaggagccacgggttcgccgggaagcagcccaagcgcatccactggtacagggcctggggcttcaccgggtacttcatccacggggtcaccgggaacgcccggatcggggacggcttcctcatcaccaggatcgtcaacaccctcgggcgcaacgggcagccccggaacccctggttcgggtacggcgtcgtcgagccccggtgcgagcccgggaacaagctcgacaggatcgcctggggcgtcacccggcacgtcgagcacaggcagccccggaacccctggatcgggaaccgcgtcgtcaagcgcctcgagc

SEQ ID NO: 44 - protein, 144 aa, Artificial Sequence
  XTEN AG144-A
GASPGTSSTGSPGSSPSASTGTGPGSSPSASTGTGPGTPGSGTASSSPGSSTPSGATGSPGSSPSASTGTGPGASPGTSSTGSPGTPGSGTASSSPGSSTPSGATGSPGTPGSGTASSSPGASPGTSSTGSPGASPGTSSTGSP

SEQ ID NO: 45 - DNA, 450 bp, Artificial Sequence
  XTEN AG144-A
ggcgcgccaggtgcctcgccgggaacatcatcaactggttcacccgggtcatccccctcggcctcaaccgggacgggtcccggctcatcccccagcgccagcactggaacaggtcctggcactcctggttccggtacggcatcgtcatccccgggaagctcaacaccgtccggagcgacaggatcacctggctcgtcaccttcggcgtcaactggaacggggccaggggcctcacccggaacgtcctcgactgggtcgcctggtacgccgggatcaggaacggcctcatcctcgcctgggtcctcaacgccctcgggtgcgactggttcgccgggaactcctggctcggggacggcctcgtcgtcgcctggggcatcaccggggacgagctccacggggtcccctggagcgtcaccggggacctcctcgacaggtagcccggcctcgagc

SEQ ID NO: 46 - protein, 144 aa, Artificial Sequence
  XTEN AG144-B
GTPGSGTASSSPGSSTPSGATGSPGASPGTSSTGSPGTPGSGTASSSPGSSTPSGATGSPGSSPSASTGTGPGSSPSASTGTGPGSSTPSGATGSPGSSTPSGATGSPGASPGTSSTGSPGASPGTSSTGSPGASPGTSSTGSP

SEQ ID NO: 47 - DNA, 450 bp, Artificial Sequence
  XTEN AG144-B
ggcgcgccaggtacaccgggcagcggcacggcttcgtcgtcacccggctcgtccacaccgtcgggagctacgggaagcccaggagcgtcaccgggaacgtcgtcaacggggtcaccgggtacgccaggtagcggcacggccagcagctcgccaggttcatcgaccccgtcgggagcgactgggtcgcccggatcaagcccgtcagcttccactggaacaggacccgggtcgtcgccgtcagcctcaacggggacaggacctggttcatcgacgccgtcaggggcgacaggctcgcccggatcgtcaacaccctcgggggcaacggggagccctggtgcgtcgcctggaacctcatccaccggaagcccgggggcctcgccgggtacgagctccacgggatcgcccggagcgtcccccggaacttcaagcacagggagccctgcctcgagc

SEQ ID NO: 48 - protein, 144 aa, Artificial Sequence
  XTEN AG144-C
GTPGSGTASSSPGASPGTSSTGSPGASPGTSSTGSPGASPGTSSTGSPGSSPSASTGTGPGTPGSGTASSSPGASPGTSSTGSPGASPGTSSTGSPGASPGTSSTGSPGSSTPSGATGSPGSSTPSGATGSPGASPGTSSTGSP

SEQ ID NO: 49 - DNA, 450 bp, Artificial Sequence
  XTEN AG144-C
ggcgcgccaggtacacccggatcgggtacagcgtcatcgagccccggtgcgtcacctggtacgtcgagcacggggtcgccaggggcgtcccctgggacgtcctcaacaggctcgcccggtgcgtcacccggcacgtcgtccacgggttcacctggtagctccccttccgcgtccactggcaccgggcctggaactccggggagcggcacagcgagctcgtcgccgggagcatcgcctgggacatcgagcaccgggtcgccaggagcatcgcccggaacatccagcacaggaagccccggcgcgtcgcccgggacatcaagcacaggttccccgggatcgagcacgccgtccggagccactggatcaccagggagctcgacaccttccggcgcaacgggatcgcccggagccagcccgggtacgtcaagcactggctcccctgcctcgagc

SEQ ID NO: 50 - protein, 144 aa, Artificial Sequence
  XTEN AG144-F
GSSPSASTGTGPGSSPSASTGTGPGASPGTSSTGSPGASPGTSSTGSPGSSTPSGATGSPGSSPSASTGTGPGASPGTSSTGSPGSSPSASTGTGPGTPGSGTASSSPGSSTPSGATGSPGSSTPSGATGSPGASPGTSSTGSP

SEQ ID NO: 51 - DNA, 450 bp, Artificial Sequence
  XTEN AG144-F
ggcgcgccaggctccagcccctccgcgagcacgggaaccggaccaggttcgtcaccctcagcatcaacggggacgggaccgggggcgtcaccaggaacgtcctccaccggctcgccgggtgcatcacccggaacgtcatcgaccggatcgccagggagctcgacgccatcaggcgcaacaggatcacctggctcaagccctagcgcgtcaaccggcacgggtccgggtgcctcccctggcacgtccagcaccggatcacccggatcgagcccatccgcctcaaccggaaccggacccggtacaccagggtcgggaacagcctcctcgtcaccaggctcctcaaccccctcgggagccacgggttcgcccggttcgtcaacgccttccggagcaactggtagccccggagcatcgccaggaacttcgagcacggggtcgcccgcctcgagc